European Patent Application EP 4 410 983 A1, published August 7, 2024. Title: 3-하이드록시프로피온산 생산 유전자가 삽입된 3-하이드록시프로피온산 생산능을 가지는 대장균 및 이의 용도. Applicant: 주식회사 엘지화학. Application WO. The sequence listing filed with the application follows.

SEQUENCE LISTING (122 sequences)

SEQ ID NO: 1 - DNA, 4107 bp, synthetic construct
  misc_feature 1..4107: note = Cas9 gene
  source 1..4107: mol_type = other DNA
atggataagaaatactcaataggcttagatatcggcacaaatagcgtcggatgggcggtgatcactgatgaatataaggttccgtctaaaaagttcaaggttctgggaaatacagaccgccacagtatcaaaaaaaatcttataggggctcttttatttgacagtggagagacagcggaagcgactcgtctcaaacggacagctcgtagaaggtatacacgtcggaagaatcgtatttgttatctacaggagattttttcaaatgagatggcgaaagtagatgatagtttctttcatcgacttgaagagtcttttttggtggaagaagacaagaagcatgaacgtcatcctatttttggaaatatagtagatgaagttgcttatcatgagaaatatccaactatctatcatctgcgaaaaaaattggtagattctactgataaagcggatttgcgcttaatctatttggccttagcgcatatgattaagtttcgtggtcattttttgattgagggagatttaaatcctgataatagtgatgtggacaaactatttatccagttggtacaaacctacaatcaattatttgaagaaaaccctattaacgcaagtggagtagatgctaaagcgattctttctgcacgattgagtaaatcaagacgattagaaaatctcattgctcagctccccggtgagaagaaaaatggcttatttgggaatctcattgctttgtcattgggtttgacccctaattttaaatcaaattttgatttggcagaagatgctaaattacagctttcaaaagatacttacgatgatgatttagataatttattggcgcaaattggagatcaatatgctgatttgtttttggcagctaagaatttatcagatgctattttactttcagatatcctaagagtaaatactgaaataactaaggctcccctatcagcttcaatgattaaacgctacgatgaacatcatcaagacttgactcttttaaaagctttagttcgacaacaacttccagaaaagtataaagaaatcttttttgatcaatcaaaaaacggatatgcaggttatattgatgggggagctagccaagaagaattttataaatttatcaaaccaattttagaaaaaatggatggtactgaggaattattggtgaaactaaatcgtgaagatttgctgcgcaagcaacggacctttgacaacggctctattccccatcaaattcacttgggtgagctgcatgctattttgagaagacaagaagacttttatccatttttaaaagacaatcgtgagaagattgaaaaaatcttgacttttcgaattccttattatgttggtccattggcgcgtggcaatagtcgttttgcatggatgactcggaagtctgaagaaacaattaccccatggaattttgaagaagttgtcgataaaggtgcttcagctcaatcatttattgaacgcatgacaaactttgataaaaatcttccaaatgaaaaagtactaccaaaacatagtttgctttatgagtattttacggtttataacgaattgacaaaggtcaaatatgttactgaaggaatgcgaaaaccagcatttctttcaggtgaacagaagaaagccattgttgatttactcttcaaaacaaatcgaaaagtaaccgttaagcaattaaaagaagattatttcaaaaaaatagaatgttttgatagtgttgaaatttcaggagttgaagatagatttaatgcttcattaggtacctaccatgatttgctaaaaattattaaagataaagattttttggataatgaagaaaatgaagatatcttagaggatattgttttaacattgaccttatttgaagatagggagatgattgaggaaagacttaaaacatatgctcacctctttgatgataaggtgatgaaacagcttaaacgtcgccgttatactggttggggacgtttgtctcgaaaattgattaatggtattagggataagcaatctggcaaaacaatattagattttttgaaatcagatggttttgccaatcgcaattttatgcagctgatccatgatgatagtttgacatttaaagaagacattcaaaaagcacaagtgtctggacaaggcgatagtttacatgaacatattgcaaatttagctggtagccctgctattaaaaaaggtattttacagactgtaaaagttgttgatgaattggtcaaagtaatggggcggcataagccagaaaatatcgttattgaaatggcacgtgaaaatcagacaactcaaaagggccagaaaaattcgcgagagcgtatgaaacgaatcgaagaaggtatcaaagaattaggaagtcagattcttaaagagcatcctgttgaaaatactcaattgcaaaatgaaaagctctatctctattatctccaaaatggaagagacatgtatgtggaccaagaattagatattaatcgtttaagtgattatgatgtcgatcacattgttccacaaagtttccttaaagacgattcaatagacaataaggtcttaacgcgttctgataaaaatcgtggtaaatcggataacgttccaagtgaagaagtagtcaaaaagatgaaaaactattggagacaacttctaaacgccaagttaatcactcaacgtaagtttgataatttaacgaaagctgaacgtggaggtttgagtgaacttgataaagctggttttatcaaacgccaattggttgaaactcgccaaatcactaagcatgtggcacaaattttggatagtcgcatgaatactaaatacgatgaaaatgataaacttattcgagaggttaaagtgattaccttaaaatctaaattagtttctgacttccgaaaagatttccaattctataaagtacgtgagattaacaattaccatcatgcccatgatgcgtatctaaatgccgtcgttggaactgctttgattaagaaatatccaaaacttgaatcggagtttgtctatggtgattataaagtttatgatgttcgtaaaatgattgctaagtctgagcaagaaataggcaaagcaaccgcaaaatatttcttttactctaatatcatgaacttcttcaaaacagaaattacacttgcaaatggagagattcgcaaacgccctctaatcgaaactaatggggaaactggagaaattgtctgggataaagggcgagattttgccacagtgcgcaaagtattgtccatgccccaagtcaatattgtcaagaaaacagaagtacagacaggcggattctccaaggagtcaattttaccaaaaagaaattcggacaagcttattgctcgtaaaaaagactgggatccaaaaaaatatggtggttttgatagtccaacggtagcttattcagtcctagtggttgctaaggtggaaaaagggaaatcgaagaagttaaaatccgttaaagagttactagggatcacaattatggaaagaagttcctttgaaaaaaatccgattgactttttagaagctaaaggatataaggaagttaaaaaagacttaatcattaaactacctaaatatagtctttttgagttagaaaacggtcgtaaacggatgctggctagtgccggagaattacaaaaaggaaatgagctggctctgccaagcaaatatgtgaattttttatatttagctagtcattatgaaaagttgaagggtagtccagaagataacgaacaaaaacaattgtttgtggagcagcataagcattatttagatgagattattgagcaaatcagtgaattttctaagcgtgttattttagcagatgccaatttagataaagttcttagtgcatataacaaacatagagacaaaccaatacgtgaacaagcagaaaatattattcatttatttacgttgacgaatcttggagctcccgctgcttttaaatattttgatacaacaattgatcgtaaacgatatacgtctacaaaagaagttttagatgccactcttatccatcaatccatcactggtctttatgaaacacgcattgatttgagtcagctaggaggtgactga

SEQ ID NO: 2 - DNA, 1885 bp, synthetic construct
  misc_feature 1..1885: note = RED recomgbinase gene
  source 1..1885: mol_type = other DNA
atggatattaatactgaaactgagatcaagcaaaagcattcactaaccccctttcctgttttcctaatcagcccggcatttcgcgggcgatattttcacagctatttcaggagttcagccatgaacgcttattacattcaggatcgtcttgaggctcagagctgggcgcgtcactaccagcagctcgcccgtgaagagaaagaggcagaactggcagacgacatggaaaaaggcctgccccagcacctgtttgaatcgctatgcatcgatcatttgcaacgccacggggccagcaaaaaatccattacccgtgcgtttgatgacgatgttgagtttcaggagcgcatggcagaacacatccggtacatggttgaaaccattgctcaccaccaggttgatattgattcagaggtataaaacgaatgagtactgcactcgcaacgctggctgggaagctggctgaacgtgtcggcatggattctgtcgacccacaggaactgatcaccactcttcgccagacggcatttaaaggtgatgccagcgatgcgcagttcatcgcattactgatcgttgccaaccagtacggccttaatccgtggacgaaagaaatttacgcctttcctgataagcagaatggcatcgttccggtggtgggcgttgatggctggtcccgcatcatcaatgaaaaccagcagtttgatggcatggactttgagcaggacaatgaatcctgtacatgccggatttaccgcaaggaccgtaatcatccgatctgcgttaccgaatggatggatgaatgccgccgcgaaccattcaaaactcgcgaaggcagagaaatcacggggccgtggcagtcgcatcccaaacggatgttacgtcataaagccatgattcagtgtgcccgtctggccttcggatttgctggtatctatgacaaggatgaagccgagcgcattgtcgaaaatactgcatacactgcagaacgtcagccggaacgcgacatcactccggttaacgatgaaaccatgcaggagattaacactctgctgatcgccctggataaaacatgggatgacgacttattgccgctctgttcccagatatttcgccgcgacattcgtgcatcgtcagaactgacacaggccgaagcagtaaaagctcttggattcctgaaacagaaagccgcagagcagaaggtggcagcatgacaccggacattatcctgcagcgtaccgggatcgatgtgagagctgtcgaacagggggatgatgcgtggcacaaattacggctcggcgtcatcaccgcttcagaagttcacaacgtgatagcaaaaccccgctccggaaagaagtggcctgacatgaaaatgtcctacttccacaccctgcttgctgaggtttgcaccggtgtggctccggaagttaacgctaaagcactggcctggggaaaacagtacgagaacgacgccagaaccctgtttgaattcacttccggcgtgaatgttactgaatccccgatcatctatcgcgacgaaagtatgcgtaccgcctgctctcccgatggtttatgcagtgacggcaacggccttgaactgaaatgcccgtttacctcccgggatttcatgaagttccggctcggtggtttcgaggccataaagtcagcttacatggcccaggtgcagtacagcatgtgggtgacgcgaaaaaatgcctggtactttgccaactatgacccgcgtatgaagcgtgaaggcctgcattatgtcgtgattgagcgggatgaaaagtacatggcgagttttgacgagatcgtgccggagttcatcgaaaaaatggacgaggcactggctgaaattggttttgtatttggggagcaatggcgatga

SEQ ID NO: 3 - DNA, 20 bp, synthetic construct
  misc_feature 1..20: note = ldhA_gRNA1
  source 1..20: mol_type = other DNA
gcacgttgtggcaggcagac

SEQ ID NO: 4 - DNA, 20 bp, synthetic construct
  misc_feature 1..20: note = ldhA_gRNA2
  source 1..20: mol_type = other DNA
taacgtctgattcagagaac

SEQ ID NO: 5 - DNA, 20 bp, synthetic construct
  misc_feature 1..20: note = ldhA_gRNA3
  source 1..20: mol_type = other DNA
aacgtctgattcagagaaca

SEQ ID NO: 6 - DNA, 20 bp, synthetic construct
  misc_feature 1..20: note = yqhD_gRNA1
  source 1..20: mol_type = other DNA
actttcctgctggcggttgg

SEQ ID NO: 7 - DNA, 20 bp, synthetic construct
  misc_feature 1..20: note = yqhD_gRNA2
  source 1..20: mol_type = other DNA
caccaaatttatcgccgcag

SEQ ID NO: 8 - DNA, 20 bp, synthetic construct
  misc_feature 1..20: note = glpK_gRNA1
  source 1..20: mol_type = other DNA
attgtctgggaaaaagaaac

SEQ ID NO: 9 - DNA, 20 bp, synthetic construct
  misc_feature 1..20: note = glpK_gRNA2
  source 1..20: mol_type = other DNA
cgtcgttcttccgaagtata

SEQ ID NO: 10 - DNA, 20 bp, synthetic construct
  misc_feature 1..20: note = gldA_gRNA1
  source 1..20: mol_type = other DNA
atcgcggagactgcgcagtg

SEQ ID NO: 11 - DNA, 20 bp, synthetic construct
  misc_feature 1..20: note = gldA_gRNA2
  source 1..20: mol_type = other DNA
cctcgatactgccaaagcac

SEQ ID NO: 12 - DNA, 20 bp, synthetic construct
  misc_feature 1..20: note = mgsA_gRNA1
  source 1..20: mol_type = other DNA
cgagataacgctgataatcg

SEQ ID NO: 13 - DNA, 20 bp, synthetic construct
  misc_feature 1..20: note = mgsA_gRNA2
  source 1..20: mol_type = other DNA
cgcagcaaggctttcacgtc

SEQ ID NO: 14 - DNA, 20 bp, synthetic construct
  misc_feature 1..20: note = poxB_gRNA1
  source 1..20: mol_type = other DNA
cagtgcatggttgccccttc

SEQ ID NO: 15 - DNA, 20 bp, synthetic construct
  misc_feature 1..20: note = poxB_gRNA2
  source 1..20: mol_type = other DNA
gtacttgtgggatctgctcc

SEQ ID NO: 16 - DNA, 20 bp, synthetic construct
  misc_feature 1..20: note = nfrA_gRNA1
  source 1..20: mol_type = other DNA
cgcatgcagccaccagtaga

SEQ ID NO: 17 - DNA, 20 bp, synthetic construct
  misc_feature 1..20: note = nfrA_gRNA2
  source 1..20: mol_type = other DNA
ccagtcgcgccattaaagtc

SEQ ID NO: 18 - DNA, 255 bp, synthetic construct
  misc_feature 1..255: note = ldhA_upstream
  source 1..255: mol_type = other DNA
ggcgattgggatgtgtgcattacccaacggcaaacgctgtagcgaacagtcacttgccgccgggagctgtggcagctattaattcattaaatccgccagcttataagttaatgtctgttttgcggtcgccagcgttaactggttcgcggtcagatccacttgtgcaccttctttcagcatttcgctaatggtgttatcgagttcattaagctgcgggttagcgcacatcatacgggtcattgccagccctttggc

SEQ ID NO: 19 - DNA, 255 bp, synthetic construct
  misc_feature 1..255: note = ldhA_downstream
  source 1..255: mol_type = other DNA
tactagcgcagcttaagctcaaagccaaaggactcgttcacctgttgcaggtacttcttgtcgtactgttttgtgctataaacggcgagtttcataagactttctccagtgatgttgaatcacatttaagctactaaaaatattttacaaaatttcaaatttaattgaaagctatggcgatattgaaaaattcatcaacaactatgcttagtgtaggcgcaaccttcaactgaacggttaaacatgccacaatac

SEQ ID NO: 20 - DNA, 255 bp, synthetic construct
  misc_feature 1..255: note = yqhD_upstream
  source 1..255: mol_type = other DNA
ggcggagttaatcccgctggctgccatcgacggctggaaatgctcatcttcgccaatgtccatcaacagttcctgtaactgcaaaatatcgacattgagacgcaaccctgccagcggcacctctgacgtggcataggtttcgcactcaaacggcaacggcaccgtcagcagcaggtattcattggcatcataacgaaacacgcgttcattgatataaccgattttatgcccggaaaagagaattatgatgccagg

SEQ ID NO: 21 - DNA, 255 bp, synthetic construct
  misc_feature 1..255: note = yqhD_downstream
  source 1..255: mol_type = other DNA
tactagcgcagcttagaacagtatgttaccaaaccggttgatgccaaaattcaggaccgtttcgcagaaggcattttgctgacgctaatcgaagatggtccgaaagccctgaaagagccagaaaactacgatgtgcgcgccaacgtcatgtgggcggcgactcaggcgctgaacggtttgattggcgctggcgtaccgcaggactgggcaacgcatatgctgggccacgaactgactgcgatgcacggtctggat

SEQ ID NO: 22 - DNA, 255 bp, synthetic construct
  misc_feature 1..255: note = glpK_upstream
  source 1..255: mol_type = other DNA
ccgggttgttgattttcttcggtgtgggttgcgttgcagcactaaaagtcgctggtgcgtcttttggtcagtgggaaatcagtgtcatttggggactgggggtggcaatggccatctacctgaccgcaggggtttccggcgcgcatcttaatcccgctgttaccattgcattgtggctgtttgcctgtttcgacaagcgcaaagttattccttttatcgtttcacaagttgccggcgctttctgtgctgcggctt

SEQ ID NO: 23 - DNA, 255 bp, synthetic construct
  misc_feature 1..255: note = glpK_downstream
  source 1..255: mol_type = other DNA
tactagcgcagcttaacctatggcactggctgctttatgctgatgaacactggcgagaaagcggtgaaatcagaaaacggcctgctgaccaccatcgcctgcggcccgactggcgaagtgaactatgcgttggaaggtgcggtgtttatggcaggcgcatccattcagtggctgcgcgatgaaatgaagttgattaacgacgcctacgattccgaatatttcgccaccaaagtgcaaaacaccaatggtgtgtat

SEQ ID NO: 24 - DNA, 255 bp, synthetic construct
  misc_feature 1..255: note = gldA_upstream
  source 1..255: mol_type = other DNA
catgcacgaagaattccgtaacgcgctggttaacgccgcctctgccgacgctatcgccagcctgctgcaacatgaactggaactgtaaaaggaaacatcatggaactgtatctggacaccgctaacgtcgcagaagtcgaacgtctggcacgcatattccccattgccggggtgacaactaacccgagcattatcgctgccagcaaggagtccatatgggaagtgctgccgcgtctgcaaaaagcgattggtgat

SEQ ID NO: 25 - DNA, 255 bp, synthetic construct
  misc_feature 1..255: note = gldA_downstream
  source 1..255: mol_type = other DNA
tactagcgcagcttagaagcggcatgtgcagaaggtgaaaccattcacaacatgcctggcggcgcgacgccagatcaggtttacgccgctctgctggtagccgaccagtacggtcagcgtttcctgcaagagtgggaataacctactccaaactcccggcttgtccgggagtttgaacgcaaaattgcctgatgcgctacgcttatcaggcctacgcaatctctgcaatatattgaatttgcgtgcttttgtagg

SEQ ID NO: 26 - DNA, 255 bp, synthetic construct
  misc_feature 1..255: note = mgsA_upstream
  source 1..255: mol_type = other DNA
gattgtgattctggagaaaggtcgctttatcagcccgtggaagcatattctggttgatgaatttcaggatatctcgccgcagcgggcagcgttgttagcggcattacgcaagcaaaacagtcagacgacgttgttcgctgttggtgatgactggcaggcgatttaccgattcagcggtgcgcaaatgtcgctcaccaccgctttccatgaaaactttggtgaaggcgaacgctgtgatttagacacgacttaccg

SEQ ID NO: 27 - DNA, 255 bp, synthetic construct
  misc_feature 1..255: note = mgsA_downstream
  source 1..255: mol_type = other DNA
tactagcgcagcttatccgcgcaggtaaagtgcgagtcgtcagttccataatgtacatccgtagttaactttcctacagattactgtaagcacttatcgctgcaagataaagaccgaaaaagcctgcgcacaggcacaaaaatctcaggaagatggttgtttttccgcccactgcaggaaagtatttcgcgtttgtgggtcagccagtttaaaccaatacttcagccgttgttctgtgagcacctgagactgcgg

SEQ ID NO: 28 - DNA, 255 bp, synthetic construct
  misc_feature 1..255: note = poxB_upstream
  source 1..255: mol_type = other DNA
ttaccttagccagtttgttttcgccagttcgatcacttcatcaccgcgtccgctgatgattgcgcgcagcatatacaggctgaaacctttggcctgttcgagtttgatctgcggtggaatggctaactcttctttggcgaccaccacatccaccaacaccggaccgtcgatggagaaggcgcgttgcagggcttcatcaacttcagacgctttttctacacggatacccgtaatgccgcacgcttcggcaatgcg

SEQ ID NO: 29 - DNA, 255 bp, synthetic construct
  misc_feature 1..255: note = poxB_downstream
  source 1..255: mol_type = other DNA
tactagcgcagcttaagctcgcaatagtgactacattcgcggaatagctcttgtgggtgggtttcctggaaatagccgctgccaatttcgctggagggaatatgagcggcaatcgccagtaccggaacgtgattgcggtggcaatcgaacaggccgttgattaagtgcaggttgccggggccgcacgatccggcgcagaccgccagttctccgctaagttgtgcttcagcgccagcggcaaaggccgccacttct

SEQ ID NO: 30 - DNA, 255 bp, synthetic construct
  misc_feature 1..255: note = nfrA_upstream
  source 1..255: mol_type = other DNA
tgtgcggccaggcgtcgtagtgcgtctcgccggtccagatattccagcggaccccgactccgccaagctgcgcgccctgagtgcctttatcacgatagccgttgtcctgaacgtgagcgtaaggctcaatagtctgtccgttagctaccttctgatgccagctgacgcgataatctgccgtccacgcctgaatatcctggcggatatattgcgccgcatcgaggtacaggttttgggcaaaccagcctgaaccgt

SEQ ID NO: 31 - DNA, 255 bp, synthetic construct
  misc_feature 1..255: note = nfrA_downstream
  source 1..255: mol_type = other DNA
tactagcgcagcttaggcgagcagtttttgcgctgcgtcgtactgaccttcttttaacagcaccggtagcgtcgcgccaacaacatactggcggttgtcggcaaactgtaccgtataattcgccaacgcctgaacggggttagcgctgtatttagataacagatagagccaacttttctcttgtgcgtccgtggtaaatagtggcttattttcaatgagataatgctggaggcgtgctttttcgccacgataagc

SEQ ID NO: 32 - DNA, 18 bp, synthetic construct
  misc_feature 1..18: note = poxB_For
  source 1..18: mol_type = other DNA
agtgtgcgcaccagatgc

SEQ ID NO: 33 - DNA, 21 bp, synthetic construct
  misc_feature 1..21: note = poxB_Rev
  source 1..21: mol_type = other DNA
gtttgccgtccagttcgacga

SEQ ID NO: 34 - DNA, 25 bp, synthetic construct
  misc_feature 1..25: note = nfrA_For
  source 1..25: mol_type = other DNA
cgctctccgttacgttgattaatcg

SEQ ID NO: 35 - DNA, 21 bp, synthetic construct
  misc_feature 1..21: note = nfrA_Rev
  source 1..21: mol_type = other DNA
gtttgccgtccagttcgacga

SEQ ID NO: 36 - DNA, 20 bp, synthetic construct
  misc_feature 1..20: note = mgsA_For
  source 1..20: mol_type = other DNA
gaaggcagaaaacgctgtcg

SEQ ID NO: 37 - DNA, 21 bp, synthetic construct
  misc_feature 1..21: note = mgsA_Rev
  source 1..21: mol_type = other DNA
gtttgccgtccagttcgacga

SEQ ID NO: 38 - DNA, 18 bp, synthetic construct
  misc_feature 1..18: note = ldhA_For
  source 1..18: mol_type = other DNA
caatgatcggcggttcgc

SEQ ID NO: 39 - DNA, 21 bp, synthetic construct
  misc_feature 1..21: note = ldhA_Rev
  source 1..21: mol_type = other DNA
gtttgccgtccagttcgacga

SEQ ID NO: 40 - DNA, 16 bp, synthetic construct
  misc_feature 1..16: note = yqhD_For
  source 1..16: mol_type = other DNA
cacgtcgagtaaccgc

SEQ ID NO: 41 - DNA, 21 bp, synthetic construct
  misc_feature 1..21: note = yqhD_Rev
  source 1..21: mol_type = other DNA
gtttgccgtccagttcgacga

SEQ ID NO: 42 - DNA, 20 bp, synthetic construct
  misc_feature 1..20: note = gldA_For
  source 1..20: mol_type = other DNA
ctgcgggcgatcagcatatg

SEQ ID NO: 43 - DNA, 21 bp, synthetic construct
  misc_feature 1..21: note = gldA_Rev
  source 1..21: mol_type = other DNA
gtttgccgtccagttcgacga

SEQ ID NO: 44 - DNA, 23 bp, synthetic construct
  misc_feature 1..23: note = glpK_For
  source 1..23: mol_type = other DNA
gctgtttgcctgtttcgacaagc

SEQ ID NO: 45 - DNA, 21 bp, synthetic construct
  misc_feature 1..21: note = glpK_Rev
  source 1..21: mol_type = other DNA
gtttgccgtccagttcgacga

SEQ ID NO: 46 - DNA, 24 bp, synthetic construct
  misc_feature 1..24: note = 3-HP_For
  source 1..24: mol_type = other DNA
ctagatttacagctagctcagtcc

SEQ ID NO: 47 - DNA, 29 bp, synthetic construct
  misc_feature 1..29: note = 3-HP_Rev
  source 1..29: mol_type = other DNA
tgccatattaataatcgatccctatctgc

SEQ ID NO: 48 - DNA, 38 bp, synthetic construct
  misc_feature 1..38: note = ldhA_upstream_For
  source 1..38: mol_type = other DNA
actgaaccgctctaggcgattgggatgtgtgcattacc

SEQ ID NO: 49 - DNA, 34 bp, synthetic construct
  misc_feature 1..34: note = ldhA_upstream_Rev
  source 1..34: mol_type = other DNA
tagctgtaaatctagatctctctgcactgcccgc

SEQ ID NO: 50 - DNA, 36 bp, synthetic construct
  misc_feature 1..36: note = ldhA_downstream_For
  source 1..36: mol_type = other DNA
tactagcgcagcttaagctcaaagccaaaggactcg

SEQ ID NO: 51 - DNA, 39 bp, synthetic construct
  misc_feature 1..39: note = ldhA_downstream_Rev
  source 1..39: mol_type = other DNA
cagcagcctaggttaacgatcaattgcccgctattttcc

SEQ ID NO: 52 - DNA, 34 bp, synthetic construct
  misc_feature 1..34: note = yqhD_upstream_For
  source 1..34: mol_type = other DNA
actgaaccgctctagggcggagttaatcccgctg

SEQ ID NO: 53 - DNA, 40 bp, synthetic construct
  misc_feature 1..40: note = yqhD_upstream_Rev
  source 1..40: mol_type = other DNA
tagctgtaaatctagcactttctgttcgcgaaccagtttc

SEQ ID NO: 54 - DNA, 40 bp, synthetic construct
  misc_feature 1..40: note = yqhD_downstream_For
  source 1..40: mol_type = other DNA
tactagcgcagcttagaacagtatgttaccaaaccggttg

SEQ ID NO: 55 - DNA, 33 bp, synthetic construct
  misc_feature 1..33: note = yqhD_downstream_Rev
  source 1..33: mol_type = other DNA
cagcagcctaggttaagggctttgccgacacct

SEQ ID NO: 56 - DNA, 34 bp, synthetic construct
  misc_feature 1..34: note = glpK_upstream_For
  source 1..34: mol_type = other DNA
tactagcgcagcttaacctatggcactggctgct

SEQ ID NO: 57 - DNA, 40 bp, synthetic construct
  misc_feature 1..40: note = glpK_upstream_Rev
  source 1..40: mol_type = other DNA
tagctgtaaatctaggtcatattacagcgaagctttttgt

SEQ ID NO: 58 - DNA, 35 bp, synthetic construct
  misc_feature 1..35: note = glpK_downstream_For
  source 1..35: mol_type = other DNA
tactagcgcagcttaaagcgtttatgccgcatccg

SEQ ID NO: 59 - DNA, 36 bp, synthetic construct
  misc_feature 1..36: note = glpK_downstream_Rev
  source 1..36: mol_type = other DNA
cagcagcctaggttatcttcgttgtcgcctttgacg

SEQ ID NO: 60 - DNA, 37 bp, synthetic construct
  misc_feature 1..37: note = gldA_upstream_For
  source 1..37: mol_type = other DNA
actgaaccgctctagcatgcacgaagaattccgtaac

SEQ ID NO: 61 - DNA, 39 bp, synthetic construct
  misc_feature 1..39: note = gldA_upstream_Rev
  source 1..39: mol_type = other DNA
tagctgtaaatctagaaacctaaaacaaatttgtcaccc

SEQ ID NO: 62 - DNA, 35 bp, synthetic construct
  misc_feature 1..35: note = gldA_downstream_For
  source 1..35: mol_type = other DNA
tactagcgcagcttagaagcggcatgtgcagaagg

SEQ ID NO: 63 - DNA, 38 bp, synthetic construct
  misc_feature 1..38: note = gldA_downstream_Rev
  source 1..38: mol_type = other DNA
cagcagcctaggttatctgaaaccaccccaatatgtgc

SEQ ID NO: 64 - DNA, 40 bp, synthetic construct
  misc_feature 1..40: note = mgsA_upstream_For
  source 1..40: mol_type = other DNA
actgaaccgctctaggattgtgattctggagaaaggtcgc

SEQ ID NO: 65 - DNA, 38 bp, synthetic construct
  misc_feature 1..38: note = mgsA_upstream_Rev
  source 1..38: mol_type = other DNA
tagctgtaaatctagcggaccgtctgaagtaatattgc

SEQ ID NO: 66 - DNA, 33 bp, synthetic construct
  misc_feature 1..33: note = mgsA_downstream_For
  source 1..33: mol_type = other DNA
tactagcgcagcttatccgcgcaggtaaagtgc

SEQ ID NO: 67 - DNA, 39 bp, synthetic construct
  misc_feature 1..39: note = mgsA_downstream_Rev
  source 1..39: mol_type = other DNA
cagcagcctaggttacgaatgaatgagagcaaaagcggg

SEQ ID NO: 68 - DNA, 35 bp, synthetic construct
  misc_feature 1..35: note = poxB_upstream_For
  source 1..35: mol_type = other DNA
actgaaccgctctagcggcattaaagatgcgcgca

SEQ ID NO: 69 - DNA, 33 bp, synthetic construct
  misc_feature 1..33: note = poxB_upstream_Rev
  source 1..33: mol_type = other DNA
tagctgtaaatctagacaacagcgtgctgggct

SEQ ID NO: 70 - DNA, 40 bp, synthetic construct
  misc_feature 1..40: note = poxB_downstream_For
  source 1..40: mol_type = other DNA
tactagcgcagcttaagctcgcaatagtgactacattcgc

SEQ ID NO: 71 - DNA, 33 bp, synthetic construct
  misc_feature 1..33: note = poxB_downstream_Rev
  source 1..33: mol_type = other DNA
cagcagcctaggttacgtgatgacctgcggccc

SEQ ID NO: 72 - DNA, 38 bp, synthetic construct
  misc_feature 1..38: note = nfrA_upstream_For
  source 1..38: mol_type = other DNA
actgaaccgctctagtgtgcggccaggcgtcgtagtgc

SEQ ID NO: 73 - DNA, 33 bp, synthetic construct
  misc_feature 1..33: note = nfrA_upstream_Rev
  source 1..33: mol_type = other DNA
tagctgtaaatctaggggcttccggacgatccg

SEQ ID NO: 74 - DNA, 33 bp, synthetic construct
  misc_feature 1..33: note = nfrA_downstream_For
  source 1..33: mol_type = other DNA
tactagcgcagcttaggcgagcagtttttgcgc

SEQ ID NO: 75 - DNA, 40 bp, synthetic construct
  misc_feature 1..40: note = nfrA_downstream_Rev
  source 1..40: mol_type = other DNA
cagcagcctaggttaacagaaaaataacgacgaagcaacc

SEQ ID NO: 76 - DNA, 23 bp, synthetic construct
  misc_feature 1..23: note = fhuA_gRNA1
  source 1..23: mol_type = other DNA
tacggctggttgccgaaagaggg

SEQ ID NO: 77 - DNA, 23 bp, synthetic construct
  misc_feature 1..23: note = fhuA_gRNA2
  source 1..23: mol_type = other DNA
gccaaagatccggcaaactccgg

SEQ ID NO: 78 - DNA, 23 bp, synthetic construct
  misc_feature 1..23: note = fadL_gRNA1
  source 1..23: mol_type = other DNA
gcaccgattaacgaccaatttgg

SEQ ID NO: 79 - DNA, 23 bp, synthetic construct
  misc_feature 1..23: note = fadL_gRNA2
  source 1..23: mol_type = other DNA
cctgaaatgtgggaagtgtcagg

SEQ ID NO: 80 - DNA, 23 bp, synthetic construct
  misc_feature 1..23: note = adhE_gRNA
  source 1..23: mol_type = other DNA
cgggtgcggggagaagataatgg

SEQ ID NO: 81 - DNA, 23 bp, synthetic construct
  misc_feature 1..23: note = pflB_gRNA
  source 1..23: mol_type = other DNA
cattactttgtcccacagggtgg

SEQ ID NO: 82 - DNA, 23 bp, synthetic construct
  misc_feature 1..23: note = aldA_gRNA
  source 1..23: mol_type = other DNA
gattcacgcgtcattaatagtgg

SEQ ID NO: 83 - DNA, 40 bp, synthetic construct
  misc_feature 1..40: note = fhuA_upstream_For
  source 1..40: mol_type = other DNA
actgaaccgctctagtaccaacaataacgtagatacctgg

SEQ ID NO: 84 - DNA, 34 bp, synthetic construct
  misc_feature 1..34: note = fhuA_upstream_Rev
  source 1..34: mol_type = other DNA
tagctgtaaatctagagactgtcgcgccgcaata

SEQ ID NO: 85 - DNA, 37 bp, synthetic construct
  misc_feature 1..37: note = fhuA_downstream_For
  source 1..37: mol_type = other DNA
tactagcgcagcttagcaccgtctaaaggtaagcagt

SEQ ID NO: 86 - DNA, 33 bp, synthetic construct
  misc_feature 1..33: note = fhuA_downstream_Rev
  source 1..33: mol_type = other DNA
cagcagcctaggttatccgacggcggctgatga

SEQ ID NO: 87 - DNA, 36 bp, synthetic construct
  misc_feature 1..36: note = fadL_upstream_For
  source 1..36: mol_type = other DNA
actgaaccgctctagaaaacctgacccataacactc

SEQ ID NO: 88 - DNA, 40 bp, synthetic construct
  misc_feature 1..40: note = fadL_upstream_Rev
  source 1..40: mol_type = other DNA
tagctgtaaatctaggaccataacctcaatgatttatttt

SEQ ID NO: 89 - DNA, 34 bp, synthetic construct
  misc_feature 1..34: note = fadL_downstream_For
  source 1..34: mol_type = other DNA
tactagcgcagcttacgattcactatagcctggc

SEQ ID NO: 90 - DNA, 40 bp, synthetic construct
  misc_feature 1..40: note = fadL_downstream_Rev
  source 1..40: mol_type = other DNA
cagcagcctaggttaattaacttcatcattgttattttca

SEQ ID NO: 91 - DNA, 33 bp, synthetic construct
  misc_feature 1..33: note = adhE_upstream_For
  source 1..33: mol_type = other DNA
actgaaccgctctagaaagcgcagcgccagctc

SEQ ID NO: 92 - DNA, 37 bp, synthetic construct
  misc_feature 1..37: note = adhE_upstream_Rev
  source 1..37: mol_type = other DNA
tagctgtaaatctagacaacggcgtaatctgtgcttc

SEQ ID NO: 93 - DNA, 38 bp, synthetic construct
  misc_feature 1..38: note = adhE_downstream_For
  source 1..38: mol_type = other DNA
tactagcgcagcttacttgctcttgagtgaaactggca

SEQ ID NO: 94 - DNA, 36 bp, synthetic construct
  misc_feature 1..36: note = adhE_downstream_Rev
  source 1..36: mol_type = other DNA
cagcagcctaggttataacgcgtaccccagacgatg

SEQ ID NO: 95 - DNA, 40 bp, synthetic construct
  misc_feature 1..40: note = pflB_upstream_For
  source 1..40: mol_type = other DNA
actgaaccgctctagcagtgatgtactgtttagccagcca

SEQ ID NO: 96 - DNA, 40 bp, synthetic construct
  misc_feature 1..40: note = pflB_upstream_Rev
  source 1..40: mol_type = other DNA
tagctgtaaatctaggtaaatctggtgttctgaccggtct

SEQ ID NO: 97 - DNA, 39 bp, synthetic construct
  misc_feature 1..39: note = pflB_downstream_For
  source 1..39: mol_type = other DNA
tactagcgcagcttagtaacacctaccttcttaagtgga

SEQ ID NO: 98 - DNA, 40 bp, synthetic construct
  misc_feature 1..40: note = pflB_downstream_Rev
  source 1..40: mol_type = other DNA
cagcagcctaggttaggcgagatatgatctatatcaattt

SEQ ID NO: 99 - DNA, 35 bp, synthetic construct
  misc_feature 1..35: note = aldA_upstream_For
  source 1..35: mol_type = other DNA
actgaaccgctctagatgcaccacgctggttaagt

SEQ ID NO: 100 - DNA, 37 bp, synthetic construct
  misc_feature 1..37: note = aldA_upstream_Rev
  source 1..37: mol_type = other DNA
tagctgtaaatctagtattaccggtcaaaagagcggg

SEQ ID NO: 101 - DNA, 33 bp, synthetic construct
  misc_feature 1..33: note = aldA_downstream_For
  source 1..33: mol_type = other DNA
tactagcgcagcttaaaacctttggcccggtgc

SEQ ID NO: 102 - DNA, 39 bp, synthetic construct
  misc_feature 1..39: note = aldA_downstream_Rev
  source 1..39: mol_type = other DNA
cagcagcctaggttaggtgcgaagaaggtgttgatttcc

SEQ ID NO: 103 - DNA, 850 bp, synthetic construct
  misc_feature 1..850: note = fhuA_upstream
  source 1..850: mol_type = other DNA
taccaacaataacgtagatacctggtttgcgggcattgacggcagcacggtgaccatcacctgggtcggccgtgataacaaccagccgaccaaactgtatggtgccagcggggcaatgtcgatttatcagcgttatctggctaaccagacgccaacgccgctgaatcttgttccgccagaagatattgcagatatgggcgtggactacgacggcaactttgtttgcagcggtggcatgcgtatcttgccggtctggaccagcgatccgcaatcgctgtgccagcagagcgagatgcagcagcagccgtcaggcaatccgtttgatcagtcttctcagccgcagcaacagccgcaacagcaacctgctcagcaagagcagaaagacagcgacggtgtagccggttggatcaaggatatgtttggtagtaattaacatctaagcgtgaaataccggatggcgagttgccatccggtaaaataacatcccatctaagatattaaccctttcttttcatctggttgtttattaacccttcaggaacgctcagattgcgtaccgcttgcgaacccgccagcgtttcgaatattatcttatctttataataatcattctcgtttacgttatcattcactttacatcagagatataccaatggcgcgttccaaaactgctcagccaaaacactcactgcgtaaaatcgcagttgtagtagccacagcggttagcggcatgtctgtttatgcacaggcagcggttgaaccgaaagaagacactatcaccgttaccgctgcacctgcgccgcaagaaagcgcatgggggcctgctgcaactattgcggcgcgacagtct

SEQ ID NO: 104 - DNA, 850 bp, synthetic construct
  misc_feature 1..850: note = fhuA_downstream
  source 1..850: mol_type = other DNA
gcaccgtctaaaggtaagcagtatgaagtcggcgtgaaatatgtaccggaagatcgtccgattgtagttactggtgccgtgtataatctcactaaaaccaacaacctgatggcggaccctgagggttccttcttctcggttgaaggtggcgagatccgcgcacgtggcgtagaaatcgaagcgaaagcggcgctgtcggcgagtgttaacgtagtcggttcttatacttacaccgatgcggaatacaccaccgatactacctataaaggcaatacgcctgcacaggtgccaaaacacatggcttcgttgtgggctgactacaccttctttgacggtccgctttcaggtctgacgctgggcaccggtggtcgttatactggctccagttatggtgatccggctaactcctttaaagtgggaagttatacggtcgtggatgcgttagtacgttatgatctggcgcgagtcggcatggctggctccaacgtggcgctgcatgttaacaacctgttcgatcgtgaatacgtcgccagctgctttaacacttatggctgcttctggggcgcagaacgtcaggtcgttgcaaccgcaaccttccgtttctaatttctcttttggggcacggatttccgtgcccatttcacaagttggctgttatgcaggaatacacgaatcattccgataccacttttgcactgcgtaatatctcctttcgtgtgcccgggcgcacgcttttgcatccgctgtcgttaacctttcctgccgggaaagtgaccggtctgattggtcacaacggttctggtaaatccactctgctcaaaatgcttggccgtcatcagccgccgtcgga

SEQ ID NO: 105 - DNA, 850 bp, synthetic construct
  misc_feature 1..850: note = fadL_upstream
  source 1..850: mol_type = other DNA
aaaacctgacccataacactcccctgtaaaaaaataaataaagtggtctgacctgatcatagtcttaaccatttttttacatttagccaagtggagaaaagggaaagtgggagctatgacacagagagaaaagaagaagagaaaagaaaacgcccctgccagcaactgacaggggcgtacgtacccgagaggaattaacgcagacccagctggaaaatcagcatttcagcttcgcaggcaaaagtgaaatcgatatccaggcgcacaccgtcagactcttcagtgaaagtcggggtgattttgcaaggttcagattccacgctacgggctttttcagtcagcgccgccagcgtttgctctgcttctgcgcggtttgcaaacacgcggctgtaagacgcggtgcagtcggagttgtccataatggtgccaacatccatacagcagcaaaccggggtttcatcagcactacatttactcatcgttgatttcctctgtatgtgcacccaaggtgccagataaacgttgtggatattttacgcttccggaaagtgctgctccagttgttaattctgcaaaatcggataagtgaccgaaatcacacttaaaaatgatctaaaacaaaattcacccgaatccatgagtgcgccacctccaaattttgccagctggatcgcgtttcttagatcatatttgaaaaaagatagaaacatacttgcaacattccagctggtccgacctatactctcgccactggtctgatttctaagatgtacctcagaccctacacttcgcgctcctgttacagcacgtaacatagtttgtataaaaataaatcattgaggttatggtc

SEQ ID NO: 106 - DNA, 850 bp, synthetic construct
  misc_feature 1..850: note = fadL_downstream
  source 1..850: mol_type = other DNA
cgattcactatagcctggcttacaccagctggagtcagttccagcagctgaaagcgacctcaaccagtggcgacacgctgttccagaaacatgaaggctttaaagatgcttaccgcatcgcgttgggtaccacttattactacgatgataactggaccttccgtaccggtatcgcctttgatgacagcccagttcctgcacagaatcgttctatctccattccggaccaggaccgtttctggctgagtgcaggtacgacttacgcatttaataaagatgcttcagtcgacgttggtgtttcttatatgcacggtcagagcgtgaaaattaacgaaggcccataccagttcgagtctgaaggtaaagcctggctgttcggtactaactttaactacgcgttctgataacgcgttcgcctggataaagtcacctgcatagcaggtgactttaactcccccacttcaccgaaagtagtgtcctcattgcttacctcctgagttttgcaaacagcctgttggcagcttgccctttcaaatcaataagcggtatccacagacaaacctgaagggaaaggcatattttcaggcgttctgctcgtccttctcaaagagtttacttttctgcatttccaggatactccccccccctggctattgtgcgctcatacactcaaattaaagataggttctaaataaatgagcgttttttgatagtctatttcattaggtaatatatatttgtaacaaatcaatcaaaatggaataaaatcatgctaccatctatttcaatcaacaataccagcgcagcttacccagaatccatcaatgaaaataacaatgatgaagttaat

SEQ ID NO: 107 - DNA, 998 bp, synthetic construct
  misc_feature 1..998: note = adhE_upstream
  source 1..998: mol_type = other DNA
aaagcgcagcgccagctcttcgaagtgagtttccggatgttcgtacataacccacatgatcttcgcggcgtccatcggggaaccaccacccagcgcgataatcacgtctggtttgaaggagtttgccagttctgcacctttacgaacgatgctcagggtcgggtccgcttctacttcgaagaagacttcagtttcaacgcctgctgctttcagtacggaagtgatctgatcagcataaccattgttgaacaggaagcggtcagtcacgatgagcgcacgtttgtggccatcagtaatcacttcatccagcgcgattggcagggagccacggcggaagtagatagatttcggaagtttgtgccacaacatgttttcagctcgcttagcaacggttttcttgttgatcaggtgtttcggaccaacgttttcagagatggagttaccaccccaagaaccacaacccagagtcagggaaggtgcgagtttgaagttatacaggtcaccgataccaccctgagacgctggggtgttaatcaggatacgcgccgttttcattttctgaccgaagtaagaaacgcgagccggttggttatcctggtcagtgtacaggcaagaggtatgaccgataccgcccatagcaaccagtttctctgctttttctaccgcgtcttcgaaatctttagcgcggtacattgccagagtcggggacagtttttcatgtgcgaacggttcgctttcatcaacaacggtcacttcaccgatcagaatcttggtgttttctggtacagagaagcctgccagttcagcaattttataggctggctgaccaacgatagccgcgttcagcgcaccgtttttcaggataacatcctgaacagctttcagctctttaccctgcaacagatagccgccgtgggttgcaaaacgttcacgtacagcgtcataaacagagtcaacaacaacaacagactgttcagaagcacagattacgccgttgt

SEQ ID NO: 108 - DNA, 998 bp, synthetic construct
  misc_feature 1..998: note = adhE_downstream
  source 1..998: mol_type = other DNA
cttgctcttgagtgaaactggcatattcacgctgggctttttttacacgctctacgagtgcgttaagttcagcgacattagtaacagccataatgctctcctgataatgttaaacttttttagtaaatcatctgctcgaatacgagagtatagtcagtgcggtgatgatttgcttaacctatgaaaatcaaaagcttactcgcgctcacactcactgtgatttactaaaagagtttaaacattagagttattatctctaatgcgtcacttccaggtggcgtaagcaagattactcacttctgggtactgattacgtgatccaaatcaaatttttgcaaagctgacacctttcagcatcgcttttcgccattatagctaacagttaataaattgtagtatgatttggtggctacattagcatgttttgcacaactagataacaataacgaatgatagcaattttaagtagttaggaggtgaaaaatgctgtcaaaaggcgtattgtcagcgcgtcttttcaaccttatttatggctaacattatccggcttttgcttcggagctaaccgtgattcagaccttttttgattttcccgtttacttcaaatttttcatcgggttatttgcgctggtcaacccggtagggattattcccgtctttatcagcatgaccagttatcagacagcggcagcgcgaaacaaaactaaccttacagccaacctgtctgtggccattatcttgtggatctcgctttttctcggcgacacgattctacaactttttggtatatcaattgattcgttccgtatcgccgggggtatcctggtggtgacaatagcgatgtcgatgatcagcggcaagcttggcgaggataaacagaacaagcaagaaaaatcagaaaccgcggtacgtgaaagcattggtgtggtgccactggcgttgccgttgatggcggggccaggggcgatcagttctaccatcgtctggggtacgcgtta

SEQ ID NO: 109 - DNA, 999 bp, synthetic construct
  misc_feature 1..999: note = pflB_upstream
  source 1..999: mol_type = other DNA
cagtgatgtactgtttagccagccagtccatgaagtgatccatgcgctccatcacttcatcatagttcaggacatcgcctttgatcggttcagacttcggaccaacctgcattttcagtttttcgtcaacgccgccgttgattgcgtacagcatggttttcgccaggtttgcacgcgcaccgaagaactgcatttgtttaccaacgatcatcgggcttacgcagcaagcaatagcgtagtcatcgttgttgaagtccggacgcatcaggtcatcgttctcatactgcagagaagaggtgtcgatggacactttagcggcgaatttcttgaagttcagcggcagtttttcagaccacagaatggtcatgttcggttccggagacggacccatggtgtacagggtgttcaggaaacggaagctgtttttggtaaccagggtacgaccgtcgaggcccataccaccgatagattcggttgcccagatcgggtcgccagagaacagttcatcgtattccggagtacgcaggaagcgaaccatacgcagtttcatgaccaggtggtcaaccatttcctgcgcttcttgttcggtgatcttgccagctttcaggtcacgttcgatgtacacatccaggaaggtggaggtacgaccgaaggacattgcagcaccgttctgagacttaacagcagccaggtagccgaagtaagtccactggatagcttcctgagcgttggtagccggaccagagatgtcgtagccgtatttcgcagccatttctttcatctgacccagagcgcggtgctgttcagcgatttcttcgcgcagacggatagtctgttccaggtttacgccgttttccagatcagcctgcagagaagtgaactgtgccagtttgtctttcatcaggtagtcgataccgtacagcgcaacgcgacggtagtcaccgatgatacggccacggccatatgcatctggcagaccggtcagaacaccagatttac

SEQ ID NO: 110 - DNA, 994 bp, synthetic construct
  misc_feature 1..994: note = pflB_downstream
  source 1..994: mol_type = other DNA
gtaacacctaccttcttaagtggattttttatttactgcgtacttcgacaaccattaatggtggtcgttttcacgcaggtaaatgacccagtatgtcaacccaaccaacaaaccaccaccgataatgttgccgatcgtaaccggaatcaggttatcagtgatgaaattcatcacggtcaggtgagaaaaattttccggtgcagaaccgactgcggtccaaaattccggggatgcgaagtcgcggattacaatacccatcgggatcataaacatgtttgcgatactgtgctcaaaaccgctggcaacaaacatcgcgaccggcagcaccataatgaacgctttgtccatcaggctgcggccagaataactcatccatactgccagacataccatcaggtttgccaggataccaagacagacggcctcaataaaagtatggtgcactttgtggtcggcggtttgtaggacgtttagtccccattgaccatttgcggtcatatactcgccggaaagccacattaaaagtacaaacagcagtgcgccgaccaggttgccaaaatagacatttagccagtttttcgccaactgaccccaggtgatgcgcccactcgccttagcaacaacaatcaacacggtggaagtaaagagatcggctccgcagacaacacaaagaatcagccccagagagaagcaaatgccgccaaccagttttgccatgccgaagggcattgtgcctgtgccagtggttgctgtgatatagaagacgaatgcgattgagatgaaaacaccggcggtaatcgccagatagaaagtcttaagcggatgtttcgttgctttatagacacccgcctcttcggccactttggccattgcagcaggaagtaaaagatcaaaagggttgtcagctttcacactaactctctctttattaagtcggcgacgagatactaacaaagcattatagatgagaaattgatatagatcatatctcgcc

SEQ ID NO: 111 - DNA, 997 bp, synthetic construct
  misc_feature 1..997: note = aldA_upstream
  source 1..997: mol_type = other DNA
atgcaccacgctggttaagttatcccggattcgttcctcagttaggaaataacgcagacagtgtaatctttattaatcagttacaaggattatggccagttgagcgttatctctcactactcactggcgagctgccgcgtttacgcgatgatagcgatggctacggtccccgcgggcgagattttatcgttcacgttgattttccggcagaagtcatccatgcatggcaaacgctgaaacatgatgcggtgctcatcgaggcgatggaaagtcgctcgttacgttaaaaattgcccgtttgtgaaccacttgtttgcaaacgggcatgactcctgacttttatttctgccttttattccttttacacttgtttttatgaagcccttcacagaattgtcctttcacgattccgtctctctgatgattgatgttaattaacaatgtattcaccgaaaacaaacatataaatcacaggagtcgcccatgtcagtacccgttcaacatcctatgtatatcgatggacagtttgttacctggcgtggagacgcatggattgatgtggtaaaccctgctacagaggctgtcatttcccgcatacccgatggtcaggccgaggatgcccgtaaggcaatcgatgcagcagaacgtgcacaaccagaatgggaagcgttgcctgctattgaacgcgccagttggttgcgcaaaatctccgccgggatccgcgaacgcgccagtgaaatcagtgcgctgattgttgaagaagggggcaagatccagcagctggctgaagtcgaagtggcttttactgccgactatatcgattacatggcggagtgggcacggcgttacgagggcgagattattcaaagcgatcgtccaggagaaaatattcttttgtttaaacgtgcgcttggtgtgactaccggcattctgccgtggaacttcccgttcttcctcattgcccgcaaaatggctcccgctcttttgaccggtaata

SEQ ID NO: 112 - DNA, 999 bp, synthetic construct
  misc_feature 1..999: note = aldA_downstream
  source 1..999: mol_type = other DNA
aaacctttggcccggtgctgccagttgtcgcatttgacacgctggaagatgctatctcaatggctaatgacagtgattacggcctgacctcatcaatctatacccaaaatctgaacgtcgcgatgaaagccattaaagggctgaagtttggtgaaacttacatcaaccgtgaaaacttcgaagctatgcaaggcttccacgccggatggcgtaaatccggtattggcggcgcagatggtaaacatggcttgcatgaatatctgcagacccaggtggtttatttacagtcttaatgagtgaaagaggcggaggttttttcctccgcctgtgcgcgtcagagtttagcgaatttttcgagggtgcgaataagctgtgtgacgaagccatattcgttatcgtaccaggcgaccgttttcaccagttgtaaatcgcccacggcggtaatttccgtttgcgtggcatcaaacaccgaaccgaaatggctgccaatgatatcggaagagactatttcttcatcggtataaccaaatgactcgttattggtggttgcttgtttaagtgcgttattcacctcttcggcagtcacttttttccgagaatcgataccagttcagtgaccgaacctgttttcaccggcacgcgttgcgcatgacctttcagtttgccgctcagttccgggatcaccagaccaatggcttttgccgcccccgtagtgtggggaatgatattttctgccgctgcgcgtgaagcacgtaaatctttaccacgcgggccatccaccagtgactgggtgccagtataggcatgaatggtcgtcatcgtgccgacttctatcccgaaactgtcatgcaaggctttggccatcggcgcaagacagttagtggtgcatgacgccacggaaacaatggtgtcgttgccatccagagtgtcgtcattgacgttataaacgatagttttcatttcaccggcaggggcggaaatcaacaccttcttcgcacc

SEQ ID NO: 113 - DNA, 25 bp, synthetic construct
  misc_feature 1..25: note = fhuA_For
  source 1..25: mol_type = other DNA
tggaccatgcagcaggtggtacaac

SEQ ID NO: 114 - DNA, 21 bp, synthetic construct
  misc_feature 1..21: note = fhuA_Rev
  source 1..21: mol_type = other DNA
gtttgccgtccagttcgacga

SEQ ID NO: 115 - DNA, 25 bp, synthetic construct
  misc_feature 1..25: note = fadL_For
  source 1..25: mol_type = other DNA
gtacgtaaaccgctaacaatggcga

SEQ ID NO: 116 - DNA, 21 bp, synthetic construct
  misc_feature 1..21: note = fadL_Rev
  source 1..21: mol_type = other DNA
gtttgccgtccagttcgacga

SEQ ID NO: 117 - DNA, 25 bp, synthetic construct
  misc_feature 1..25: note = adhE_For
  source 1..25: mol_type = other DNA
ttcgggaacttgtagatacgtttac

SEQ ID NO: 118 - DNA, 21 bp, synthetic construct
  misc_feature 1..21: note = adhE_Rev
  source 1..21: mol_type = other DNA
gtttgccgtccagttcgacga

SEQ ID NO: 119 - DNA, 23 bp, synthetic construct
  misc_feature 1..23: note = pflB_For
  source 1..23: mol_type = other DNA
gtacttgtcgtgcatgtagtgga

SEQ ID NO: 120 - DNA, 21 bp, synthetic construct
  misc_feature 1..21: note = pflB_Rev
  source 1..21: mol_type = other DNA
gtttgccgtccagttcgacga

SEQ ID NO: 121 - DNA, 18 bp, synthetic construct
  misc_feature 1..18: note = aldA_For
  source 1..18: mol_type = other DNA
gttccgccgtatgactgg

SEQ ID NO: 122 - DNA, 21 bp, synthetic construct
  misc_feature 1..21: note = aldA_Rev
  source 1..21: mol_type = other DNA
gtttgccgtccagttcgacga